European Patent Specification EP 3 592 763 B1, published February 25, 2026. Title: COMPOSITIONS, METHODS, AND SYSTEMS FOR AFFINITY-BASED. Applicant: Recombipure. The sequence listing filed with the application follows.

SEQUENCE LISTING (94 sequences)

SEQ ID NO: 1 - protein, 7 aa, Artificial Sequence
  recombinant
GHHHHHH

SEQ ID NO: 2 - protein, 19 aa, Artificial Sequence
  recombinant
KIANFIPAELKLITKANVQ

SEQ ID NO: 3 - protein, 276 aa, Artificial Sequence
  recombinant
MGSSCHHHHHHSQDPNSSSMKEGKTIGLVISTLNNPFFVTLKNGAEEKAKELGYKIIVEDSQNDSSKELSNVEDLIQQKVDVLLINPVDSDAVVTAIKEANSKNIPVITIDRSANGGDVVSHIASDNVKGGEMAAEFIAKALKGKGNVVELEGIPGASAARDRGKGFDEAIAKYPDIKIVAKQAADFDRSKGLSVMENILQAQPKIDAVFAQNDEMALGAIKAIEAANRQGIIVVGFDGTEDALKAIKEGKMAATIAQQPALMGSLGVEMADKYLK

SEQ ID NO: 4 - protein, 285 aa, Artificial Sequence
  recombinant
MGSSGEKIPNFIPAELKLITKENVQGSENLYFQGGSMVSKGEELIKENMHMKLYMEGTVNNHHFKCTSEGEGKPYEGTQTMRIKVVEGGPLPFAFDILATSFMYGSRTFINHTQGIPDFFKQSFPEGFTWERVTTYEDGGVLTATQDTSLQDGCLIYNVKIRGVNFPSNGPVMQKKTLGWEANTEMLYPADGGLEGRSDMALKLVGGGHLICNFKTTYRSKKPAKNLKMPGVYYVDHRLERIKEADKETYVEQHEVAVARYCDLPSKLGHKLNGSSGHHHHHHHH

SEQ ID NO: 5 - protein, 529 aa, Artificial Sequence
  recombinant
MGSSSQDPNSSSMKEGKTIGLVISTLNNPFFVTLKNGAEEKAKELGYKIIVEDSQNDSSKELSNVEDLIQQKVDVLLINPVDSDAVVTAIKEANSKNIPVITIDRSANGGDVVSHIASDNVKGGEMAAEFIAKALKGKGNVVELEGIPGASAARDRGKGFDEAIAKYPDIKIVAKQAADFDRSKGLSVMENILQAQPKIDAVFAQNDEMALGAIKAIEAANRQGIIVVGFDGTEDALKAIKEGKMAATIAQQPALMGSLGVEMADKYLKGSENLYFQGGSMVSKGEELIKENMHMKLYMEGTVNNHHFKCTSEGEGKPYEGTQTMRIKVVEGGPLPFAFDILATSFMYGSRTFINHTQGIPDFFKQSFPEGFTWERVTTYEDGGVLTATQDTSLQDGCLIYNVKIRGVNFPSNGPVMQKKTLGWEANTEMLYPADGGLEGRSDMALKLVGGGHLICNFKTTYRSKKPAKNLKMPGVYYVDHRLERIKEADKETYVEQHEVAVARYCDLPSKLGHKLNGSSGHHHHHHHH

SEQ ID NO: 6 - protein, 287 aa, Artificial Sequence
  recombinant
MGSSHHHHHHHHGSMVSKGEELIKENMHMKLYMEGTVNNHHFKCTSEGEGKPYEGTQTMRIKVVEGGPLPFAFDILATSFMYGSRTFINHTQGIPDFFKQSFPEGFTWERVTTYEDGGVLTATQDTSLQDGCLIYNVKIRGVNFPSNGPVMQKKTLGWEANTEMLYPADGGLEGRSDMALKLVGGGHLICNFKTTYRSKKPAKNLKMPGVYYVDHRLERIKEADKETYVEQHEVAVARYCDLPSKLGHKLNGSSGENLYFQGGSGEKIPNFIPAELKLITKENVQGS

SEQ ID NO: 7 - protein, 529 aa, Artificial Sequence
  recombinant
MGSSHHHHHHHHGSMVSKGEELIKENMHMKLYMEGTVNNHHFKCTSEGEGKPYEGTQTMRIKVVEGGPLPFAFDILATSFMYGSRTFINHTQGIPDFFKQSFPEGFTWERVTTYEDGGVLTATQDTSLQDGCLIYNVKIRGVNFPSNGPVMQKKTLGWEANTEMLYPADGGLEGRSDMALKLVGGGHLICNFKTTYRSKKPAKNLKMPGVYYVDHRLERIKEADKETYVEQHEVAVARYCDLPSKLGHKLNGSSGENLYFQGGSSQDPNSSSMKEGKTIGLVISTLNNPFFVTLKNGAEEKAKELGYKIIVEDSQNDSSKELSNVEDLIQQKVDVLLINPVDSDAVVTAIKEANSKNIPVITIDRSANGGDVVSHIASDNVKGGEMAAEFIAKALKGKGNVVELEGIPGASAARDRGKGFDEAIAKYPDIKIVAKQAADFDRSKGLSVMENILQAQPKIDAVFAQNDEMALGAIKAIEAANRQGIIVVGFDGTEDALKAIKEGKMAATIAQQPALMGSLGVEMADKYLK

SEQ ID NO: 8 - protein, 273 aa, Artificial Sequence
  recombinant
MGSSPAELKLITKGSENLYFQGGSMVSKGEELIKENMHMKLYMEGTVNNHHFKCTSEGEGKPYEGTQTMRIKVVEGGPLPFAFDILATSFMYGSRTFINHTQGIPDFFKQSFPEGFTWERVTTYEDGGVLTATQDTSLQDGCLIYNVKIRGVNFPSNGPVMQKKTLGWEANTEMLYPADGGLEGRSDMALKLVGGGHLICNFKTTYRSKKPAKNLKMPGVYYVDHRLERIKEADKETYVEQHEVAVARYCDLPSKLGHKLNGSSGHHHHHHHH

SEQ ID NO: 9 - protein, 283 aa, Artificial Sequence
  recombinant
MGSSKIANFIPAELKLITKANVQGSENLYFQGGSMVSKGEELIKENMHMKLYMEGTVNNHHFKCTSEGEGKPYEGTQTMRIKVVEGGPLPFAFDILATSFMYGSRTFINHTQGIPDFFKQSFPEGFTWERVTTYEDGGVLTATQDTSLQDGCLIYNVKIRGVNFPSNGPVMQKKTLGWEANTEMLYPADGGLEGRSDMALKLVGGGHLICNFKTTYRSKKPAKNLKMPGVYYVDHRLERIKEADKETYVEQHEVAVARYCDLPSKLGHKLNGSSGHHHHHHHH

SEQ ID NO: 10 - protein, 479 aa, Artificial Sequence
  recombinant
MGSPAELKLITKGGSEQKLISEEDLGGSMRECISIHVGQAGVQIGNACWELYCLEHGIQPDGQMPSDKTIGGGDDSFNTFFSETGAGKHVPRAVFVDLEPTVIDEVRTGTYRQLFHPEQLITGKEDAANNYARGHYTIGKEIIDLVLDRIRKLADQCTGLQGFLVFHSFGGGTGSGFTSLLMERLSVDYGKKSKLEFSIYPAPQVSTAVVEPYNSILTTHTTLEHSDCAFMVDNEAIYDICRRNLDIERPTYTNLNRLIGQIVSSITASLRFDGALNVDLTEFQTNLVPYPRIHFPLATYAPVISAEKAYHEQLSVAEITNACFEPANQMVKCDPRHGKYMACCLLYRGDVVPKDVNAAIATIKTKRTIQFVDWCPTGFKVGINYQPPTVVPGGDLAKVQRAVCMLSNTTAIAEAWARLDHKFDLMYAKRAFVHWYVGEGMEEGEFSEAREDMAALEKDYEEVGVDSVEGEGEEEGEEY

SEQ ID NO: 11 - protein, 127 aa, Artificial Sequence
  recombinant
MGSSHHHHHHHHENLYFQSLGSLTIAEPAMIAECKTRTEVFEISRRLIDRTNANFLVWPPCVEVQRCSGCCNNRNVQCRPTQVQLRPVQVRKIEIVRKKPIFKKATVTLEDHLACKCETVAAARPVT

SEQ ID NO: 12 - protein, 16 aa, Artificial Sequence
  recombinant
GSLGSLTIAEPAMIAE

SEQ ID NO: 13 - protein, 21 aa, Artificial Sequence
  recombinant
GEKIPNFIPAELKLITKENVQ

SEQ ID NO: 14 - protein, 21 aa, Artificial Sequence
  recombinant
AEKIPNFIPAELKLITKENVQ

SEQ ID NO: 15 - protein, 21 aa, Artificial Sequence
  recombinant
GAKIPNFIPAELKLITKENVQ

SEQ ID NO: 16 - protein, 21 aa, Artificial Sequence
  recombinant
GEAIPNFIPAELKLITKENVQ

SEQ ID NO: 17 - protein, 21 aa, Artificial Sequence
  recombinant
GEKAPNFIPAELKLITKENVQ

SEQ ID NO: 18 - protein, 21 aa, Artificial Sequence
  recombinant
GEKIANFIPAELKLITKENVQ

SEQ ID NO: 19 - protein, 21 aa, Artificial Sequence
  recombinant
GEKIPAFIPAELKLITKENVQ

SEQ ID NO: 20 - protein, 21 aa, Artificial Sequence
  recombinant
GEKIPNAIPAELKLITKENVQ

SEQ ID NO: 21 - protein, 21 aa, Artificial Sequence
  recombinant
GEKIPNFAPAELKLITKENVQ

SEQ ID NO: 22 - protein, 21 aa, Artificial Sequence
  recombinant
GEKIPNFIAAELKLITKENVQ

SEQ ID NO: 23 - protein, 21 aa, Artificial Sequence
  recombinant
GEKIPNFIPAALKLITKENVQ

SEQ ID NO: 24 - protein, 21 aa, Artificial Sequence
  recombinant
GEKIPNFIPAEAKLITKENVQ

SEQ ID NO: 25 - protein, 21 aa, Artificial Sequence
  recombinant
GEKIPNFIPAELALITKENVQ

SEQ ID NO: 26 - protein, 21 aa, Artificial Sequence
  recombinant
GEKIPNFIPAELKAITKENVQ

SEQ ID NO: 27 - protein, 21 aa, Artificial Sequence
  recombinant
GEKIPNFIPAELKLATKENVQ

SEQ ID NO: 28 - protein, 21 aa, Artificial Sequence
  recombinant
GEKIPNFIPAELKLIAKENVQ

SEQ ID NO: 29 - protein, 21 aa, Artificial Sequence
  recombinant
GEKIPNFIPAELKLITAENVQ

SEQ ID NO: 30 - protein, 21 aa, Artificial Sequence
  recombinant
GEKIPNFIPAELKLITKANVQ

SEQ ID NO: 31 - protein, 21 aa, Artificial Sequence
  recombinant
GEKIPNFIPAELKLITKENVQ

SEQ ID NO: 32 - protein, 21 aa, Artificial Sequence
  recombinant
GEKIPNFIPAELKLITKENVQ

SEQ ID NO: 33 - protein, 21 aa, Artificial Sequence
  recombinant
GEKIPNFIPAELKLITKENVQ

SEQ ID NO: 34 - protein, 20 aa, Artificial Sequence
  recombinant
EKIPNFIPAELKLITKENVQ

SEQ ID NO: 35 - protein, 19 aa, Artificial Sequence
  recombinant
KIPNFIPAELKLITKENVQ

SEQ ID NO: 36 - protein, 18 aa, Artificial Sequence
  recombinant
IPNFIPAELKLITKENVQ

SEQ ID NO: 37 - protein, 17 aa, Artificial Sequence
  recombinant
PNFIPAELKLITKENVQ

SEQ ID NO: 38 - protein, 16 aa, Artificial Sequence
  recombinant
NFIPAELKLITKENVQ

SEQ ID NO: 39 - protein, 15 aa, Artificial Sequence
  recombinant
FIPAELKLITKENVQ

SEQ ID NO: 40 - protein, 14 aa, Artificial Sequence
  recombinant
IPAELKLITKENVQ

SEQ ID NO: 41 - protein, 13 aa, Artificial Sequence
  recombinant
PAELKLITKENVQ

SEQ ID NO: 42 - protein, 12 aa, Artificial Sequence
  recombinant
AELKLITKENVQ

SEQ ID NO: 43 - protein, 11 aa, Artificial Sequence
  recombinant
ELKLITKENVQ

SEQ ID NO: 44 - protein, 10 aa, Artificial Sequence
  recombinant
LKLITKENVQ

SEQ ID NO: 45 - protein, 9 aa, Artificial Sequence
  recombinant
KLITKENVQ

SEQ ID NO: 46 - protein, 8 aa, Artificial Sequence
  recombinant
LITKENVQ

SEQ ID NO: 47 - protein, 7 aa, Artificial Sequence
  recombinant
ITKENVQ

SEQ ID NO: 48 - protein, 6 aa, Artificial Sequence
  recombinant
TKENVQ

SEQ ID NO: 49 - protein, 5 aa, Artificial Sequence
  recombinant
KENVQ

SEQ ID NO: 50 - protein, 4 aa, Artificial Sequence
  recombinant
ENVQ

SEQ ID NO: 51 - protein, 20 aa, Artificial Sequence
  recombinant
GEKIPNFIPAELKLITKENV

SEQ ID NO: 52 - protein, 19 aa, Artificial Sequence
  recombinant
GEKIPNFIPAELKLITKEN

SEQ ID NO: 53 - protein, 18 aa, Artificial Sequence
  recombinant
GEKIPNFIPAELKLITKE

SEQ ID NO: 54 - protein, 17 aa, Artificial Sequence
  recombinant
GEKIPNFIPAELKLITK

SEQ ID NO: 55 - protein, 16 aa, Artificial Sequence
  recombinant
GEKIPNFIPAELKLIT

SEQ ID NO: 56 - protein, 15 aa, Artificial Sequence
  recombinant
GEKIPNFIPAELKLI

SEQ ID NO: 57 - protein, 14 aa, Artificial Sequence
  recombinant
GEKIPNFIPAELKL

SEQ ID NO: 58 - protein, 13 aa, Artificial Sequence
  recombinant
GEKIPNFIPAELK

SEQ ID NO: 59 - protein, 12 aa, Artificial Sequence
  recombinant
GEKIPNFIPAEL

SEQ ID NO: 60 - protein, 11 aa, Artificial Sequence
  recombinant
GEKIPNFIPAE

SEQ ID NO: 61 - protein, 10 aa, Artificial Sequence
  recombinant
GEKIPNFIPA

SEQ ID NO: 62 - protein, 9 aa, Artificial Sequence
  recombinant
GEKIPNFIP

SEQ ID NO: 63 - protein, 8 aa, Artificial Sequence
  recombinant
GEKIPNFI

SEQ ID NO: 64 - protein, 7 aa, Artificial Sequence
  recombinant
GEKIPNF

SEQ ID NO: 65 - protein, 6 aa, Artificial Sequence
  recombinant
GEKIPN

SEQ ID NO: 66 - protein, 5 aa, Artificial Sequence
  recombinant
GEKIP

SEQ ID NO: 67 - protein, 8 aa, Artificial Sequence
  recombinant
ELKLITKE

SEQ ID NO: 68 - protein, 8 aa, Artificial Sequence
  recombinant
ELKLITKA

SEQ ID NO: 69 - protein, 6 aa, Artificial Sequence
  recombinant
ELKLIT

SEQ ID NO: 70 - protein, 10 aa, Artificial Sequence
  recombinant
PAELKLITKE

SEQ ID NO: 71 - protein, 10 aa, Artificial Sequence
  recombinant
PAELKLITKA

SEQ ID NO: 72 - protein, 9 aa, Artificial Sequence
  recombinant
PAELKLITK

SEQ ID NO: 73 - protein, 12 aa, Artificial Sequence
  recombinant
FIPAELKLITKE

SEQ ID NO: 74 - protein, 12 aa, Artificial Sequence
  recombinant
FIPAELKLITKA

SEQ ID NO: 75 - protein, 11 aa, Artificial Sequence
  recombinant
FIPAELKLITK

SEQ ID NO: 76 - protein, 18 aa, Artificial Sequence
  recombinant
IANFIPAELKLITKANVQ

SEQ ID NO: 77 - protein, 16 aa, Artificial Sequence
  recombinant
KIPNFIPAELKLITKE

SEQ ID NO: 78 - protein, 16 aa, Artificial Sequence
  recombinant
KIPNFIPAELKLITKA

SEQ ID NO: 79 - protein, 15 aa, Artificial Sequence
  recombinant
KIPNFIPAELKLITK

SEQ ID NO: 80 - protein, 16 aa, Artificial Sequence
  recombinant
KIANFIPAELKLITKE

SEQ ID NO: 81 - protein, 16 aa, Artificial Sequence
  recombinant
KIANFIPAELKLITKA

SEQ ID NO: 82 - protein, 15 aa, Artificial Sequence
  recombinant
KIANFIPAELKLITK

SEQ ID NO: 83 - protein, 19 aa, Artificial Sequence
  recombinant
KIPNFIPAELKLITKANVQ

SEQ ID NO: 84 - protein, 19 aa, Artificial Sequence
  recombinant
KIANFIPAELKLITKANVQ

SEQ ID NO: 85 - protein, 19 aa, Artificial Sequence
  recombinant
RIANFIPAELKLITKANVQ

SEQ ID NO: 86 - protein, 19 aa, Artificial Sequence
  recombinant
AIANFIPAELKLITKANVQ

SEQ ID NO: 87 - protein, 19 aa, Artificial Sequence
  recombinant
AIANFIPAELKLITKENVQ

SEQ ID NO: 88 - protein, 19 aa, Artificial Sequence
  recombinant
KIPNFIPAELKLITKANAA

SEQ ID NO: 89 - protein, 19 aa, Artificial Sequence
  recombinant
KIANFIPAELKLITKANAA

SEQ ID NO: 90 - protein, 21 aa, Artificial Sequence
  recombinant
GEKIPNFIPAELKKITKENVQ

SEQ ID NO: 91 - protein, 24 aa, Artificial Sequence
  recombinant
GEKIPNFIPAELKLITKENVQGGC

SEQ ID NO: 92 - protein, 22 aa, Artificial Sequence
  recombinant
KIANFIPAELKLITKANVQGGC

SEQ ID NO: 93 - DNA, 828 bp, Artificial Sequence
  unknown
atgggcagcagctgccatcaccatcatcaccacagccaggatccgaattcgagctcgatgaaagagggcaaaacgattggcctggtgatctctaccctgaacaatccgttctttgtgaccctgaaaaatggtgcggaagaaaaagcgaaagaactgggttacaaaattatcgttgaagattcgcaaaatgattcctctaaagagctgtctaatgtcgaagatttgattcaacagaaagttgatgttctgctgatcaatccggtggatagcgatgcggttgttacggcgattaaagaagcgaatagcaaaaatatcccggttattaccatcgatcgcagcgcgaatggtggtgatgttgtttcccatatcgccagcgataatgttaagggtggcgaaatggccgcggaatttatcgcgaaagccctgaaaggcaaggggaatgttgtggaactggaaggtatcccgggggcgtctgcggcacgtgatcgcggcaaagggtttgatgaagccattgctaagtatccggatattaaaatcgttgcaaagcaggcggcggattttgatcgttccaaaggtctgtcagtgatggaaaacatcttgcaagcccagccgaaaattgatgcagtgtttgcgcaaaatgatgaaatggctctgggcgctatcaaagccattgaggccgcgaatcgtcaaggtattattgttgtgggctttgatgggaccgaagatgctctgaaagcgattaaagaagggaaaatggctgcgaccattgcgcagcagccggccctgatgggctcactgggtgtggagatggctgataaatacctgaaa

SEQ ID NO: 94 - protein, 278 aa, Artificial Sequence
  unknown
MKEGKTIGLVISTLNNPFFVTLKNGAEEKAKELGYKIIVEDSQNDSSKELSNVEDLIQQKVDVLLINPVDSDAVVTAIKEANSKNIPVITIDRSANGGDVVSHIASDNVKGGEMAAEFIAKALKGKGNVVELEGIPGASAARDRGKGFDEAIAKYPDIKIVAKQAADFDRSKGLSVMENILQAQPKIDAVFAQNDEMALGAIKAIEAANRQGIIVVGFDGTEDALKAIKEGKMAATIAQQPALMGSLGVEMADKYLKGEKIPNFIPAELKLITKENVQ